European Patent Application EP 4 707 385 A2, published March 11, 2026. Title: CELL SPECIFIC TRANSCRIPTIONAL REGULATORY SEQUENCES AND USES THEREOF. Applicant: VALORISATION HSJ, LIMITED PARTNERSHIP. Application EP. The sequence listing filed with the application follows.

SEQUENCE LISTING (82 sequences)

SEQ ID NO: 1 - DNA, 32 bp, synthetic construct
  misc_feature 1..32: note = Synthetic oligonucleotide
  source 1..32: mol_type = other DNA
atcatcgcggccgcgggtctgacgtgctctgt

SEQ ID NO: 2 - DNA, 30 bp, synthetic construct
  misc_feature 1..30: note = Synthetic oligonucleotide
  source 1..30: mol_type = other DNA
attcggtaccgtgggacaccagtcatctta

SEQ ID NO: 3 - DNA, 32 bp, synthetic construct
  misc_feature 1..32: note = Synthetic oligonucleotide
  source 1..32: mol_type = other DNA
atatgcggccgcgaccaggtttggccaataga

SEQ ID NO: 4 - DNA, 30 bp, synthetic construct
  misc_feature 1..30: note = Synthetic oligonucleotide
  source 1..30: mol_type = other DNA
atcaggatccgacacttgttctgggaccta

SEQ ID NO: 5 - DNA, 39 bp, synthetic construct
  misc_feature 1..39: note = Synthetic oligonucleotide
  source 1..39: mol_type = other DNA
cagggaattcgcttacttgttagcatccctctcatacgc

SEQ ID NO: 6 - DNA, 59 bp, Cytomegalovirus
  source 1..59: mol_type = other DNA
gtaggcgtgtacggtgggaggtctatataagcagagctcgtttagtgaaccgtcagatc

SEQ ID NO: 7 - DNA, 445 bp, Homo sapiens
  source 1..445: mol_type = other DNA
ctggtggtgtggagggccgggtggtgacactcagtgacaggtgaggatgtggcacggtgtggagggccgggtggtgacgctgagtgacaggtgaggatgtggcacggtgtggagggccgggtggtgacgctgagtgacaggtgaggatgtggcacggtgtggagggccgggtggtgacgctgagtgacaggtgaggatgtggcacggtgtggagggccgggtggtgacgctgagtgacaggtgaggatgtggcacggtgtggagggccgggtggtgacgctgagtgacacgtgaggatgtggcacggtgtggagggccgggtggtgacgctgagtgacaggtgaggatgtggcacggtgtggagggccgggtggtgacgctgagtgacaggtgaggatgtggcatagggaaacacatcctcgccgagcgcacagtgggagctccg

SEQ ID NO: 8 - DNA, 438 bp, Homo sapiens
  source 1..438: mol_type = other DNA
ctgaggacttctagctcttcctggatccttatatgcccatttgctattgtaaatagctatatgacgttgtgatactattccaaaccctagtcatagcaaccacatacctaatagccaagggataaccatactatcttccctttctgaagaacctttcagcaaaagatttcagggaattttaccaagaaaaccatcccatcccctcctccttccatttgacaggtggagaagtgaggcacagtgaagccagaggagcctggtcagacggtgagtcagaagtagagcagggctgcacctggtgacacctatttcctcccttgtggtttggcccctgcctcataggcttcctggaaaggtgtagcttcttcatggcttacttgttgagtaaacactgctatgagctttcaaatatttccctaggttgcaggaggttgtgtc

SEQ ID NO: 9 - DNA, 432 bp, Homo sapiens
  source 1..432: mol_type = other DNA
ctaaaaacaaacaaagccaaaaaaccatagcactttattttaaggatatttctactttaatccataaatggtttctagttcttgtattaatggcgacatcatgttccatgttttcatgaactgtgatttatcagagaagcccttgcaacggtgatctaggttgtgtcatcgcttctgcgtaacagcaaggcaaagctgcggatttatcgccgttctacccaggtttcctgttgattacggcagggtttgaggtgcggtccctggtgtttcatcatgacaagtggaggtttgcaggagaacttcataaccatctgcagaaaaggtgaagtcacatcttgagaccagctctagatatgttaccgatgggctaatggttttgatgtaaaataagtaaaaacattaaagggctagaagaagccagaggaaaagtca

SEQ ID NO: 10 - DNA, 199 bp, Homo sapiens
  source 1..199: mol_type = other DNA
gtgaaataagacacacacagaaagaaaaatatgatatgatatcggttgtatgtggagtcttgaaaaaaatcaccatagaaacagtgtaggaagatggttaccaggggcggggtaggggaaatgggaagatgtaggtcaaaaggtacgaagttgcggttagattctaatgttctagtgtgtaacataaggactatagtta

SEQ ID NO: 11 - DNA, 580 bp, Homo sapiens
  source 1..580: mol_type = other DNA
gcacattcatctctctgagaaacacctccctatgctgggaaatgtgaaagcaggtgggacaccagtcatcttagtacatcacattgtcactgccgcgaatgtgtgggacacccatcatcttaccacatcacatcgtcactgccgcgaacgtgtgggacacccatcatcttaccacatcacatcgtcactgccacgaacgtgtgggacacccatcatcttaccacatcacatcgtcactgccgcgaacgtgtgggacacccatcatcttaccacatcacatcgtcactgccgcgaacgtgtgggacacccatcatcttaccacatcacatcgtcactgccgcgaacgtgtgggacacccatcatcttaccacatcacatcgtcactgcgtgaatgtttttctgaatacatcacacatttggctccataaaatctgttttctaatctactttttaacttagtatgttggcctcaactttgcactttatttttcttcgtgactgtgtggtgctctcctctctggaggtgccttcactgaggctgcattgaagggctgtgtgggccagcgagtgctgtggtcgg

SEQ ID NO: 12 - DNA, 539 bp, Homo sapiens
  source 1..539: mol_type = other DNA
ctcttcattgaccctgagtttgaccaggtttggccaatagaagtcagaggaagtgacaggtgccagttacaagaagttccacaaccccttttagaaatcaactaaaccactgtgtgaataaagccaggttagcctgctggagaatgaggcccaattgctcccatcatctcacatgacagccaaccaaccaccagtcatgtgactgaggtcatcttggaccagccaaattccaaccaaccttttcagtagacctcagacacatgaacaaacccaactaagatcaaccaaccctagacagttctgcagagttgcccagtaacacacagaatcatgaccaataataaatgtgtactgtttgaagttgccacattgttaagtggtttgttatgccacaaaaactaactgacacatcaactctgaaacctccttggtttaatcagggtgctggcaggtacggagcaactgtgcccagggtaacattacttagtctcagaatcataattaattaaattgcaagtgacagaaatataataaaatct

SEQ ID NO: 13 - DNA, 591 bp, Homo sapiens
  source 1..591: mol_type = other DNA
tgattttaagtgaaaggtttctgaactgtatatatacaatatttcagaacagtaatttcctttgcttcatagtacggcacaacagtgtttgcacttgatgtttagcgtagccttggttttggttgttcagaagcctttgttagctctttggttgtgccaagaatatattgtttttgagtctccttgccgggcctcctcgccttcttgtcatgcacatcctgtacctgggttgtggttgtattgatttgctggggcgctgctgttgcaaatgtctggagtgaatgagaatgtgtttgtgggtgtctgccctcaccttggccactgatctgctttcagccctgaagtactgccatctgcatgaacattagggacccccagcctcccccaccacttagtaaagtaccctgcacatgtttgggattcaggaaatgtttgtagaaaggaaaaattccttatcattccttaccattctctgtcttgagtctgagtcatgattcaaacacttttgctaaaaggttttcgcttgaaaaattcatattcaggtacagatttacttttttttggtgtgtgtgagtttaagagctgcctcag

SEQ ID NO: 14 - DNA, 608 bp, Homo sapiens
  source 1..608: mol_type = other DNA
atcagaagttgcgtgggtcatgaagcccaaggccagcagttctggatgcctccatgaagctggatattgcttacttgttagcatccctctctggcaatcatcaataacctcttttcaaaagtacctccttatacaagactcttatcaactgatttcatcatttttagcactgaaaccttggtcttcctgctctctgctctgacagcatctctctgataacctgagaaatcagagtttcacccctgaaactaaacaggccattatttcctaattttaaatgatgacatgacaagccttcaccctatctgtttcttatttccttgaactctcccaccctcaccagcagccaacacaaatcacaacgcaatgcaaaggccaggccacagaacacgctgtgaatcgacagtttcagaagacgtcattcacacaatgtgcaaggcacttcctgcacagccatctctgtgcccctgcaaagggcatgtggcatgaggcagtaaaataagtatagtctgtgtttgggtatgaaaggtggtgggtggggcgtgaatacatccaagatatgctttaggactaagtcaaaagagaactgagagtgagaaagaagattg

SEQ ID NO: 15 - DNA, 392 bp, Homo sapiens
  source 1..392: mol_type = other DNA
tgggcatggtggctcatacctgtaatcctagcactttgggaggctgaggcaggtggatcacttgaggtcaggagctccagaccagcctgcccaacatgcattgcatccatagcttggctgactttcttaaaaaacaggttgatggcaagaaaagagaactgagtagatgttataaatagttaagtacaaatctatcactacttcttgcgaaaatgctcaggctgccacactgatgatgaatagatagctcgttcttcccaaactgagtgcagtagagtgttgcagtgctcagttgggtaggacagatgttggataattggggttatccaacatctctactaaaaatacaaaaattagctgtgcgtggtggaaggtgcctgtaatcccagcta

SEQ ID NO: 16 - DNA, 305 bp, Homo sapiens
  source 1..305: mol_type = other DNA
aaggaggaattgctgtctgagagggtattttgttccccagtgactgagggcagggcaggggcagggaaggcttcccctctcttctggccctagaggccctgtaaatgcactgtgcagtcactgacgtgccctcaggcagggccctggcgggaagggggctgttccaggtctaccagcttcacacccttattctattgaattctcatgaaaacaaaatctgtgaaacagctgtgatcttcattttctgatgagggaacagagcctccgtgcccccgagatcactggtatgactccaaagattttcc

SEQ ID NO: 17 - DNA, 433 bp, Homo sapiens
  source 1..433: mol_type = other DNA
gactcacacctttggccactgacccctgccccaccttctgagtggggttcagggactgtgctgagtctgtctctgggaagcagcagggtgcaggggcacactgatgagtggtgcatgtgcccaggggcaacatcagagccgtttagccaccagggcagtcaggcatggacagacgcatttgggagggggcggggccctgtgtcagctgttaacacttcagttcctgaagcagagaagtctggagttctggggaggggccagggaggcaggagagggaaacactgggagggtttagggcttggcctgtttatcaactactgtggaagtattttcactgttctgacaatccctgcaactatgtccatggacctgctgtctatccgccctgttcatcgggaggaagagatggagaaggctgccggggttctgggag

SEQ ID NO: 18 - DNA, 695 bp, Homo sapiens
  source 1..695: mol_type = other DNA
ccaaccccccttccccaccccaaactctgcttataggttcttatatgataatttaaactatatatgatattaaattagcactccaatagcaaaaataaagtgttcccacatcaccttctttgaaaatatttatttaaataggatgaaatgttattgagggcttttgtgtctagaaacagggttaattaaagatttcctgcctgctttgtgggtaggtgacactctcattgagatagcagcaatgccctatttagtggtctctcagctttctttctattcatctggtttggtagtggaattccatgggaagtttgaccctattcagtgatgagagaagcaaaatactgttgttcacctagaggctgtttgctcagaaaaacagggtgtcagagacatgggacgcaaacccagagtgacatagcgcagggacttggctcacttttctgagatctgtaaaatgtgatgtgactggctctcagaaaggaggctgaagggttcctgcccgattggttttcaaagggcaagagccccgctgctgaggagctgcggctttgttagacaaaagcccagggcagccccctcctgggctcagcgttttccccacctccccctttctcacaggcggtttccctgaaatgaaagaactgtgatgcatttgcgccttcaaaagcagtttttaaaatgcattaaaccca

SEQ ID NO: 19 - DNA, 383 bp, Homo sapiens
  source 1..383: mol_type = other DNA
tagcagggaggggaattttcctttctggtcacgtaggctgctgtcttcggcttcgattcgtaagccacctcccaagcccccattagccccaggtaggggacatcccatccccctaaacctccttcttgaactgacagttcacccctagaaggaggtgggaaaccactcagatccatctcaaagggatgcctaccagggtaggtgtgtgggaggaaggctgagcccatgctgtgttcaggggcccccccagaaggtgtcagcctggaggaacatgccccacagttataaaaggcatcattccaggagctatcatggcgtctgctaggggcagagaggaaggggaggcaggaaaggggctgagtattttggggctgtatgcttat

SEQ ID NO: 20 - DNA, 364 bp, Homo sapiens
  source 1..364: mol_type = other DNA
ggcctttcctccggggagactgtggaggtgtcccctcaggcagcaaaagcaccatcgcagccctcggtgtcaaggcctctctgagtcgcgctttgccttaccgtacctcgtttctgggctaggatattttgaaacacttttgtctattagctttatctaaaatagctaaaatatcagtctccatagaggcaaagtaagtggcactgagaagcaaaaaatccagccaatgtgcagttttctcctcctgccccctatttgtggaaatgaggcacggcccccatcttgtctgctgggtggggttctgtttaccacgcttggcagccaccgccacccaacaatctttcatttttctttctaacttcac

SEQ ID NO: 21 - DNA, 495 bp, Homo sapiens
  source 1..495: mol_type = other DNA
gagctccctggtgtggtgtctcaagcctgaagctcagaggctggagctattgcccctggctgtctcccctgaagtcactaaattccagcgttctgggtccccttgtccccagcacacaaggatgggctgctctgagcaagctcaggcaccctcactctgccacactgtgtgtgtgacttagaccccacaaggcttttctgagaaaacagctgtgacctgacagaaacccctgcagctgcacgggcctcagaatcccccgaggcgctggcccgggctgtgcctggctccctggtgggagcagaagtgcccatggcctctcctgccctcccaacagggcccctaaacaaattcccacacccaggtgagttaccaggagcgatcaggtgggccgaggacatttgcttgcttcaccttccctgtttctttagattgaaattcagcctgccccacttctcaggaagatgccacgaggctgatccccctgagcagtttgtc

SEQ ID NO: 22 - DNA, 418 bp, Homo sapiens
  source 1..418: mol_type = other DNA
tggctggcaatcctttttagccatcatatataatagctatctaactcttgatttttgtgtaacataaagcggtgtttcataatgaatcattttgtctgttcgtgttcaagtgccctatctattctatcatttgaaaagctagttatgatagtatggtttcaattgtcagacattctctttattctaaaaaaataggttgacccacatttagatgttttcctactcaaaggactttgaaagaactttttatgtaacacttagtcattgcccttttcacagtccctcttccgctgcttctaattaggctctttggtagctggaatcgtcatttccctggcatgaaggcacatggtaccaacttgttggttgcttgatttggagggtcaaatatggacttgcttcttttggtctaccttgc

SEQ ID NO: 23 - DNA, 303 bp, Homo sapiens
  source 1..303: mol_type = other DNA
ctgacaagatgcaagctcatcattttgttttgtgtcataagggcatttgcctactaattagcgttttggaaaacttccccaataatggggcccacagtctctaacactgcccctttgaagctagtgatccaaaaataatatcatttgacaaggtaatttcccaagccacgcctgaaatgtaaaacaaaaaaagcacctcactgcttaaaggtgctccaccagggaccttgggttttccaccaaaacttgcctcccccaccctgttactaaagttgacactgaatttgcctgcagtctccccca

SEQ ID NO: 24 - DNA, 183 bp, Homo sapiens
  source 1..183: mol_type = other DNA
tgagctgtcgcccttgggtacaccagtagcaaaaacactcctgtcctcctatgctgctgtgacaccacaccccacttcctcccgcgggcgtgtgacacttttcaaagaaaatacagtatttggtagtatcaatacagcaagcggaagcagcagtgctcagtccgcagtgagctaacagtttta

SEQ ID NO: 25 - DNA, 258 bp, Homo sapiens
  source 1..258: mol_type = other DNA
cagacatacagtactattttgttttttttaaaaaaggcttagtaaacacaaagaggagttacatactgaaacccacagctgatttaatttgcaaaaccacagcgttagcttgactaaagtaaagatgacacagataaaatgcaaccagaaaactgagataaaagatacaggataaataacttaagctgatggtttagcaagcaaacatcatgggtgtaacatgaagatctgagaagtgacttcggtccaggaaactca

SEQ ID NO: 26 - DNA, 278 bp, Homo sapiens
  source 1..278: mol_type = other DNA
ctaaaaattacaccttctgctcactctaatttattgctgtagaagaaagaataagtgagatatttccatttctagtgacaggtggctggcactttgaaaccttccatttcattactcaccttaatgttttcactaaaacacatgtggttttcaaacacaggaaggaaaacatggtaacctgtggttacaatttccactagaaaatagaaaaggtgtaggtcagaaagaatgtttgtggggtgttccttttttactttaaacatgaaaacccatgtcag

SEQ ID NO: 27 - DNA, 140 bp, Homo sapiens
  source 1..140: mol_type = other DNA
ttaagagaaaaaaaaaacacccatttatgtgaccagtattgtctgtcttttttttaatccaataaaactttcaactacaatcggtgctgatgtcaccatgttagcggcacacactcttgactctggtttgcacagttcac

SEQ ID NO: 28 - DNA, 192 bp, Homo sapiens
  source 1..192: mol_type = other DNA
cggcggaggagggaaagccgagcgccaggaaaagctcctatttgcagcacacctacccccaccgtgtgccaggcactcatcataaatgtcacaatgacagatgaggaaaccgcggctcagaaggtcaagtggctgccggaggctggcagggagcagggtggggctctgactcgggctgtgttctttcccaca

SEQ ID NO: 29 - DNA, 528 bp, Homo sapiens
  source 1..528: mol_type = other DNA
tgaaaaccacagaggaacggcgagaaggaatgggagggaggaaaatacattccgtggcagtgaagttattgaagtgccagagccaaagaacagataatttaaggaaaaaattctgtggcatctcccatcctacacataaatcactgttctctattttctgaacacgagcctatgcagggcctaggagagtccatgtgtgaaactgaatacagaatatacgacgatgtaagacgtacaacgcgcacgtatgaactatgtgtgaataggtagcgacgtaggtatcgctgagaagagaaactacaatttgagatcccacctgtggttacagaaaagcagacagagccctcgatgaattaaatgcagaatgcatcagaaatgtggcagtacagaaacgccccgcagacgaggaaatcctaaatctgttgtctgcatctctctaagaaaaagaacctacaaggtaaagaaacagtcctcacaaagccggtcccagaaaccattaattacactttagaaagaaataggagttta

SEQ ID NO: 30 - DNA, 897 bp, Homo sapiens
  source 1..897: mol_type = other DNA
aatttcaaactcattttctaattcaaaagaaacacagatgaatttaaaaattagcagaggtcacacgtgcctgttcgcaagcacccctcctcctcagcttcgtcttttgccaagactatgtaccagcactttttcctttctctcctcttttttttatttttttatttttggtaacatctggtattctttcctttttttggcagtctctgccttttcactttcctcatgcagcagccctgcgagcccccgtaattgagtttgaaggtgtccaaagccgtttgctgtgctgcagctctgatttctgcgtcaagtcctaacagccaaccaacctgggagccaggccctgttggcgtccccgagacagccccgggattatccaggcctccagggctcagttctgagctgggatctccacgtcccagaccagagatccaactcactgcctctaagggagtctgggaggaaaagaaacaaacaaaaaatatctccttcccctcccactttcagcgttgaaagttaaacccctgagatgacagggtgttcacccgattccaaagaacggggtttcctctccccaccacccaggctgtggcgctgtgccttggcctgctgtgtgcgacacttcccaggaaggtagcaaggtcaccctcaacatcaggcagcagagtcacccccagccccaaatttctgggtcagagtaagtggaccaagtgggcctgaaagctcacgttcaaggcctttgtagacacccccaaagactgtggtttcacttccgctggcaggcagataccaagctaggcgtgtagggtgcctgcatatgtgtgcatgtgtccctccttagaactgtatcgataatggaagaaataaaaggagaaagccaagccctgggaagggcaa

SEQ ID NO: 31 - DNA, 526 bp, Homo sapiens
  source 1..526: mol_type = other DNA
tggctcctatgctgggttttcaggggaggggagaaccactttatatatttatttatttatttaaattttttaaaatataacataaatattcggctctcggccgcccggcagccagtcctctgcggtgactgggcgcgcagccctctcgagctccgcgcgggcagcccggccccagcccggcgaggtgcgcggcggattgcaagcatataacctgcccgcggtctcgatggcacccagaggatgttttatttctattgcagttaaaaaaaaaaaaaaaaaaaaaaaaaaaaaaaaaaaggaacggcgacccaggcaccgcgagagaaagaacggcggggaaatgttcgcgcgcagcgaagaagccgccccgcgggctgcggcgggcggggagcgccgcaaagccaccttcccggtgcaagtgtgcggggactcggggcgggttcccctgcaaacaccgtacctggcccgctcgcgctcgcttttcccctctgctaaataaacccaacagggacggtggaagctgctg

SEQ ID NO: 32 - DNA, 189 bp, Homo sapiens
  source 1..189: mol_type = other DNA
cagctagtgggtggtggatccgtgctcttgaccaccccactctgttgcctttctgttagacaacaccttgtctactttctcttccccatttcacagatgaggagacaggaccggaactgtgaggacaatctgtctatagttaggcagtgagctgactgcagactcaggctctcctgggaccctcttcag

SEQ ID NO: 33 - DNA, 438 bp, Homo sapiens
  source 1..438: mol_type = other DNA
gcaaaaaggcaggggctgcaggggactttataaagttgtgctgtctgggctgaaggcttgcagacaggaagcttgggtgcaggtgggctgtgagctgaatgcttgcaacaggatgtttgggtgctagtgagctgtttgctgttgaccctatttctcagaacattcactcccctctacccctgtgtctgttcttgccagctaagctcatttccaattttcttttagctccttagggctccacatgcgtgacttattagaggagcaaaagaagccgaatatggaaggggaaagccttggcctgatccagggtgctctagaacaaattcctcccactgaactgtcctgctgtggggcaagcaggtgagcacttgttctgttgtcagtcaccatttgcccccggggtggggtgtaacctgccaggcatcctcaagggatgca

SEQ ID NO: 34 - DNA, 301 bp, Homo sapiens
  source 1..301: mol_type = other DNA
cccccaggctggtatttcagtgacactcttagtctgttgttgtcccaaatgctgcgtacctgaaagaaagagcaccccttttgaggcatcaagacttgattcagtctcagttctgagactgaatcaacaactttcaacaggtgaataataagaacctcagaaacctgcgctgacgccctcagaagctggtttcccgtcctctgtggaagtggatttagaagccagttgagcagccatgtgaccttgaacaagtcacttctgtgttctgcactgtgagctctattccactggcccctttcta

SEQ ID NO: 35 - DNA, 342 bp, Homo sapiens
  source 1..342: mol_type = other DNA
tgaacccaagactctacaacatcctggcctcgatttttggtccagctctggttggttctttctgtgttattctgttctgctcctcaattcctctcccctcccctccccctcctctccccaccccttcccccaccccctccccctcccctcttctgtcaccttgcactgtgcactttaatgcacattgcactatgtcaaggtactaactttgacaactgctctcataattccaaccacattcaggctgagggttgcagcttggctccccctcactcttctcaccttcaccacacaggacattggctgtgcacagccacttgtttattgcagctggagaccaca

SEQ ID NO: 36 - DNA, 99 bp, Homo sapiens
  source 1..99: mol_type = other DNA
cttgctggctctcctcggtggcttcctcttgaatgaacctttcttctgaaggcttgatttccttccgggaggcttagtgtttctgctcagccttctttc

SEQ ID NO: 37 - DNA, 658 bp, Homo sapiens
  source 1..658: mol_type = other DNA
tctgtcactccctcgttgcggactcctatgtaggtcgcctggtgtggggagaagcattctttgtggtattcggttgggtagaagccaatcacagcttccacctacactcaaggggagggagttgtacagggtgtaagcaatttggggagtcaccttagaattctgcccaccacagtacctttctggttatttcatggacttccgttcccaagaaatctgagcgtttgcgtcctaggaagactggtgagagcagccccagtggaggaataaaaactaagatctggaaaatcagcagtgggttgttttcatctctcagcaggcaggaaacaggaggagaaaggaatgtctgtaggctcccaacactgatgggaaggaggtgtttggctggggtagagctccgcaggaatctcccaggctcctctagctaggtgcagccgtgttttatccggctgtctttacatgggctgatcactcaggagtggcatatggcaggagcacgctttggggtacgagcctcctggagaatgaactgcagcacacaagccagacagatggtggcttagtcccccttggacaagagtgtgtcctgcacactggagggcggggtgctgagaggcgcttgtggtgtctgaggccgagctttgctgagttcacctga

SEQ ID NO: 38 - DNA, 351 bp, Homo sapiens
  source 1..351: mol_type = other DNA
tgaaagaaagagaataaagcactgggctttgcaaactaggctaaggccccaaaccacaagattatcttgatgcatgtgattgggaaggaggactaattagaagagaggatgtcattttattttctaaccagccctctctgatctgaagccatgacaccccctcacttgttacctagcaacccttctttgtatatgtaaggttacttcattcctgcattgttattcaatttatttgccattttaagtgtcttgatcctctctaggatcaccctggtgtgattggctggcattagtctctaaaataccggagggcagtctattaagtggatccaaatgtcattgtacagctca

SEQ ID NO: 39 - DNA, 153 bp, Homo sapiens
  source 1..153: mol_type = other DNA
ctgagatgttcgtagtattgtcatctacatttcatagaagaagaaactgaaacaggttaggtaacttactcgtggtcacagaggtaattggtggatttgaggattcacaggattctaaaatcgagttgctgcactgccttctttaaaaaatta

SEQ ID NO: 40 - DNA, 210 bp, Homo sapiens
  source 1..210: mol_type = other DNA
tgtcagccagtggggtggcagcccctttgtacagagcaccatgggggttggggtggggaggataaggcaacatgtcaaacccatcaaggaggctttgtgaccccagtgatattttttgcagaacgtggtggattttcgatgtgaccacaatgacatccgccttgcagtggcagaacagatgcaattgcacaagttctggagaaactttct

SEQ ID NO: 41 - DNA, 154 bp, Homo sapiens
  source 1..154: mol_type = other DNA
tgctctctgcttaccaaactcctctcccttaagacccagctcaagcatctccttcctgtggggtttagctccttccccctcccactcccagacagtacagaccacatccttctcttctctgtgtcacccggaccttgggtatctgcagactgga

SEQ ID NO: 42 - DNA, 165 bp, Homo sapiens
  source 1..165: mol_type = other DNA
taacttaagcgtgttggtatctctgttagtggtgaagtcggctgcaaaccacaaaacacctgactgctacggaagatattaacagggacttttttccttctgcataacaggaagtcttgagtaggtagtcgaggttgggtagaggacacttctgtttcaattcta

SEQ ID NO: 43 - DNA, 391 bp, Homo sapiens
  source 1..391: mol_type = other DNA
gcattgctcagaattgctcgactttgattataattatcctacgatcgataaggatccaggtgtacgtaacataacactgtatcacattatttaaatcaggtccttttcattaagctgtgtctgttggtgctggctagtttattggtgtgtgtgggtgtgtgggggtgtgtgtgtgtgtgtgttagaaacttgtaactatagtttcagttttctggcctattatattcctactgtctttgtatgtttgttttgtatgattcttattattttcaccagaagcggaaaccctttttaagctgaaaaaggatgattcatttcgtacacagtgagggccctcttaccttatttatttgctcacatattaatagaggagacagtttttcatgcagtg

SEQ ID NO: 44 - DNA, 281 bp, Homo sapiens
  source 1..281: mol_type = other DNA
ttctgcatgagcaggccccgctgaaaaggaaggcggctcgccagatttgtttcgaattatgaaaatagatgttgtctccccaccacatctgttttgcctgacaaatgagcagcagctcgcctcctaaataaggcagcacaccaagacggtcttgaaactccggcttctccaactcttcagaaaaggagaagaagaagaaaaaagagtccaagcctcccaggtttgagctctaaaagccagacctttttcaatgtcatctctcacgccgcagtctccggggg

SEQ ID NO: 45 - DNA, 118 bp, Homo sapiens
  source 1..118: mol_type = other DNA
tattaacaagtttgtggtaaggtgttatgacaatgatagaaaactaatacacggggatttcccaagactctcaagtgattgttcattttccttttaggttctttttttttttttttga

SEQ ID NO: 46 - DNA, 500 bp, Homo sapiens
  source 1..500: mol_type = other DNA
gccggctctgtcgtcgaggcgctcacaggcaggcacacgtgagctcctggaggacagggagagcggccgccccgcccctgcggagcacaggacgcttcctgccacccctgcagagcatgggacgcttcctgccatggtgccgtggcaatgggtggcacctgcctgtggccccttctcagaaggacgttttaaacgcgtgaggtctgatgcacagccacagggagacacagacgagcagatgtgggcatccgagtatttacaaggtctggtggctcctgcagccgcgacacgggctgagcgcaagtgatgtgtgaggtgtccccaacagatggcacggggagcgcccacacccgccaccgcggggtctgcggaagctcgtgtcagctggaggttagggaagacgcacaggggctcattctccacccaggttcaaactccctgaactcacgagacccaggctgaagacatggacagactcccagccccagcgcccctctgac

SEQ ID NO: 47 - DNA, 155 bp, Homo sapiens
  source 1..155: mol_type = other DNA
ctgactgataaaagaaaaacaaattttccttcaaggcagtatgataacaatctcttaaccactgggaggaatgtttatgacattcatctctgagctgtgaactgccaaaatgaggcacgcctagcaacataacctggccgaccctaggccgcgag

SEQ ID NO: 48 - DNA, 81 bp, Homo sapiens
  source 1..81: mol_type = other DNA
gtacttatataagggggtgggggcgcgttcgtcctcagtcgcgatcgaacactcgagccgagcagacgtgcctacggaccg

SEQ ID NO: 49 - DNA, 76 bp, Homo sapiens
  source 1..76: mol_type = other DNA
caacaaaatgtcgtaacaagggcggtaggcgtgtacggtgggaggtctatataagcagagctcgtttagtgaaccg

SEQ ID NO: 50 - DNA, 31 bp, Homo sapiens
  source 1..31: mol_type = other DNA
agagggtatataatggaagctcgacttccag

SEQ ID NO: 51 - DNA, 63 bp, Homo sapiens
  source 1..63: mol_type = other DNA
ttcgcatattaaggtgacgcgtgtggcctcgaacaccgagcgaccctgcagcgacccgcttaa

SEQ ID NO: 52 - DNA, 203 bp, Homo sapiens
  source 1..203: mol_type = other DNA
tgcatctcaattagtcagcaaccatagtcccgcccctaactccgcccatcccgcccctaactccgcccagttccgcccattctccgccccatcgctgactaattttttttatttatgcagaggccgaggccgcctcggcctctgagctattccagaagtagtgaggaggcttttttggaggcctaggcttttgcaaaaagctt

SEQ ID NO: 53 - DNA, 41 bp, Homo sapiens
  source 1..41: mol_type = other DNA
ggggggctataaaagggggtgggggcgttcgtcctcactct

SEQ ID NO: 54 - DNA, 178 bp, Homo sapiens
  source 1..178: mol_type = other DNA
ctgacaaattcagtataaaagcttggggctggggccgagcactggggactttgagggtggccaggccagcgtaggaggccagcgtaggatcctgctgggagcggggaactgagggaagcgacgccgagaaagcaggcgtaccacggagggagagaaaagctccggaagcccagcagcg

SEQ ID NO: 55 - DNA, 25 bp, Homo sapiens
  source 1..25: mol_type = other DNA
tctagagggtatataatgggggcca

SEQ ID NO: 56 - DNA, 32 bp, synthetic construct
  misc_feature 1..32: note = Synthetic oligonucleotide
  source 1..32: mol_type = other DNA
tattcagcggccgcacctgggtcagtgcgtca

SEQ ID NO: 57 - DNA, 28 bp, synthetic construct
  misc_feature 1..28: note = Synthetic oligonucleotide
  source 1..28: mol_type = other DNA
gtacgaattcgagagcaccacacagtca

SEQ ID NO: 58 - DNA, 28 bp, synthetic construct
  misc_feature 1..28: note = Synthetic oligonucleotide
  source 1..28: mol_type = other DNA
gcgactagttgccagcaccctgattaaa

SEQ ID NO: 59 - DNA, 36 bp, synthetic construct
  misc_feature 1..36: note = Synthetic oligonucleotide
  source 1..36: mol_type = other DNA
cgcgcgaattcaccatactggtatattcattctctc

SEQ ID NO: 60 - DNA, 32 bp, synthetic construct
  misc_feature 1..32: note = Synthetic oligonucleotide
  source 1..32: mol_type = other DNA
ggccgctgacttagtcctaaagcatatcttgg

SEQ ID NO: 61 - DNA, 40 bp, synthetic construct
  misc_feature 1..40: note = Synthetic oligonucleotide
  source 1..40: mol_type = other DNA
acggcaatcttggtaccctccagtgccagatttttcaggg

SEQ ID NO: 62 - DNA, 47 bp, synthetic construct
  misc_feature 1..47: note = Synthetic oligonucleotide
  source 1..47: mol_type = other DNA
catgcgggtaccagtacgactagtgaactggctgggctattttgtgc

SEQ ID NO: 63 - DNA, 50 bp, Homo sapiens
  source 1..50: mol_type = other DNA
ggtgtggagggccgggtggtgacrctsagtgacaggtgaggatgtggcay

SEQ ID NO: 64 - DNA, 50 bp, Homo sapiens
  source 1..50: mol_type = other DNA
cggtgtggagggccgggtggtgacgctgagtgacaggtgaggatgtggca

SEQ ID NO: 65 - DNA, 41 bp, Homo sapiens
  source 1..41: mol_type = other DNA
gtgggacacccatcatcttaccacatcacatcgtcactgcc

SEQ ID NO: 66 - DNA, 21 bp, Homo sapiens
  source 1..21: mol_type = other DNA
yscctyccccwccycytycch

SEQ ID NO: 67 - DNA, 15 bp, Homo sapiens
  misc_feature 9: note = n is a, c, g, or t
  source 1..15: mol_type = other DNA
aaaadaaanaaarwa

SEQ ID NO: 68 - DNA, 20 bp, Homo sapiens
  source 1..20: mol_type = other DNA
ytggkggshrggsgkstgtg

SEQ ID NO: 69 - DNA, 45 bp, Homo sapiens
  misc_feature 12: note = n is a, c, g, or t
  misc_feature 24: note = n is a, c, g, or t
  source 1..45: mol_type = other DNA
ctcvgvscdggndgcchggchmanvccgggccwgbbbcgcggvsg

SEQ ID NO: 70 - DNA, 11 bp, Homo sapiens
  source 1..11: mol_type = other DNA
tcwstkttctg

SEQ ID NO: 71 - DNA, 14 bp, Homo sapiens
  source 1..14: mol_type = other DNA
gtgdmasgtgcctg

SEQ ID NO: 72 - DNA, 21 bp, Homo sapiens
  source 1..21: mol_type = other DNA
gcagccrccycrckgkctgag

SEQ ID NO: 73 - DNA, 29 bp, Homo sapiens
  source 1..29: mol_type = other DNA
cccctgcrgagcayrggacgcttcctgcc

SEQ ID NO: 74 - DNA, 15 bp, Homo sapiens
  source 1..15: mol_type = other DNA
tgkcctctmcccacm

SEQ ID NO: 75 - DNA, 21 bp, Homo sapiens
  source 1..21: mol_type = other DNA
gccytbhtgtyasrcamaasm

SEQ ID NO: 76 - DNA, 37 bp, Homo sapiens
  source 1..37: mol_type = other DNA
swmtgacacmctgtgkgtgtgmsyywgmmsycasywg

SEQ ID NO: 77 - DNA, 21 bp, Homo sapiens
  source 1..21: mol_type = other DNA
acytkctgcwcwgccttmttt

SEQ ID NO: 78 - DNA, 11 bp, Homo sapiens
  source 1..11: mol_type = other DNA
cggggagcgcc

SEQ ID NO: 79 - DNA, 19 bp, Homo sapiens
  source 1..19: mol_type = other DNA
agghagcavagkcaccctc

SEQ ID NO: 80 - DNA, 36 bp, Homo sapiens
  misc_feature 17: note = n is a, c, g, or t
  misc_feature 19: note = n is a, c, g, or t
  source 1..36: mol_type = other DNA
tbtggcgagbcdccttngnhttcwgygbgcchcact

SEQ ID NO: 81 - DNA, 11 bp, Homo sapiens
  source 1..11: mol_type = other DNA
tgtgcccaggg

SEQ ID NO: 82 - DNA, 11 bp, Homo sapiens
  source 1..11: mol_type = other DNA
gaggtgtcccc